European Patent Application EP 4 786 595 A1, published August 5, 2026. Title: SIRNA FOR INHIBITING HEPATITIS B VIRUS AND USE THEREOF. Applicant: Beijing Kawin Technology Share-Holding Co., Ltd. Application EP. The sequence listing filed with the application follows.

SEQUENCE LISTING (52 sequences)

SEQ ID NO: 1 - RNA, 19 nt, synthetic construct
  source 1..19: mol_type = other RNA
  modified_base 8: mod_base = OTHER; note; note (original language) = 2'-methoxy
  modified_base 9..10: mod_base = OTHER; note; note (original language) = 2'-deoxy-2'-fluoro
  modified_base 1..6: mod_base = OTHER; note; note (original language) = 2'-methoxy
  modified_base 7: mod_base = OTHER; note; note (original language) = 2'-deoxy-2'-fluoro
  modified_base 11..19: mod_base = OTHER; note; note (original language) = 2'-methoxy
  modified_base 1..2: mod_base = OTHER; note; note (original language) = 3'-phosphorothioate
tgtgcactccgcttcacca

SEQ ID NO: 2 - RNA, 19 nt, synthetic construct
  source 1..19: mol_type = other RNA
  modified_base 1..6: mod_base = OTHER; note; note (original language) = 2'-methoxy
  modified_base 10..19: mod_base = OTHER; note; note (original language) = 2'-methoxy
  modified_base 7..9: mod_base = OTHER; note; note (original language) = 2'-deoxy-2'-fluoro
  modified_base 1..2: mod_base = OTHER; note; note (original language) = 3'-phosphorothioate
tgtgcactccgcttcacca

SEQ ID NO: 3 - RNA, 21 nt, synthetic construct
  source 1..21: mol_type = other RNA
  modified_base 13: mod_base = OTHER; note; note (original language) = hypoxanthine
  modified_base 1: mod_base = OTHER; note; note (original language) = 2'-methoxy
  modified_base 3..5: mod_base = OTHER; note; note (original language) = 2'-methoxy
  modified_base 7: mod_base = OTHER; note; note (original language) = 2'-methoxy
  modified_base 9..11: mod_base = OTHER; note; note (original language) = 2'-methoxy
  modified_base 13: mod_base = OTHER; note; note (original language) = 2'-methoxy
  modified_base 15: mod_base = OTHER; note; note (original language) = 2'-methoxy
  modified_base 17: mod_base = OTHER; note; note (original language) = 2'-methoxy
  modified_base 19..21: mod_base = OTHER; note; note (original language) = 2'-methoxy
  modified_base 2: mod_base = OTHER; note; note (original language) = 2'-deoxy-2'-fluoro
  modified_base 6: mod_base = OTHER; note; note (original language) = 2'-deoxy-2'-fluoro
  modified_base 8: mod_base = OTHER; note; note (original language) = 2'-deoxy-2'-fluoro
  modified_base 12: mod_base = OTHER; note; note (original language) = 2'-deoxy-2'-fluoro
  modified_base 14: mod_base = OTHER; note; note (original language) = 2'-deoxy-2'-fluoro
  modified_base 16: mod_base = OTHER; note; note (original language) = 2'-deoxy-2'-fluoro
  modified_base 18: mod_base = OTHER; note; note (original language) = 2'-deoxy-2'-fluoro
  modified_base 1..2: mod_base = OTHER; note; note (original language) = 3'-phosphorothioate
  modified_base 19..20: mod_base = OTHER; note; note (original language) = 3'-phosphorothioate
  modified_base 13: mod_base = OTHER; note; note (original language) = N=hypoxanthine
tggtgaagcgaantgcacagg

SEQ ID NO: 4 - RNA, 21 nt, synthetic construct
  source 1..21: mol_type = other RNA
  modified_base 1..2: mod_base = OTHER; note; note (original language) = 3'-phosphorothioate
  modified_base 19..20: mod_base = OTHER; note; note (original language) = 3'-phosphorothioate
  modified_base 1: mod_base = OTHER; note; note (original language) = 2'-methoxy
  modified_base 3..5: mod_base = OTHER; note; note (original language) = 2'-methoxy
  modified_base 7: mod_base = OTHER; note; note (original language) = 2'-methoxy
  modified_base 9..11: mod_base = OTHER; note; note (original language) = 2'-methoxy
  modified_base 13: mod_base = OTHER; note; note (original language) = 2'-methoxy
  modified_base 15: mod_base = OTHER; note; note (original language) = 2'-methoxy
  modified_base 17: mod_base = OTHER; note; note (original language) = 2'-methoxy
  modified_base 19..21: mod_base = OTHER; note; note (original language) = 2'-methoxy
  modified_base 2: mod_base = OTHER; note; note (original language) = 2'-deoxy-2'-fluoro
  modified_base 6: mod_base = OTHER; note; note (original language) = 2'-deoxy-2'-fluoro
  modified_base 12: mod_base = OTHER; note; note (original language) = 2'-deoxy-2'-fluoro
  modified_base 14: mod_base = OTHER; note; note (original language) = 2'-deoxy-2'-fluoro
  modified_base 16: mod_base = OTHER; note; note (original language) = 2'-deoxy-2'-fluoro
  modified_base 18: mod_base = OTHER; note; note (original language) = 2'-deoxy-2'-fluoro
  modified_base 1: mod_base = OTHER; note; note (original language) = 5'-vinylphosphonate
  modified_base 13: mod_base = OTHER; note; note (original language) = N=hypoxanthine
tggtgaagcgaantgcacagg

SEQ ID NO: 5 - RNA, 21 nt, synthetic construct
  source 1..21: mol_type = other RNA
  modified_base 1: mod_base = OTHER; note; note (original language) = 3'-phosphorothioate
  modified_base 1: mod_base = OTHER; note; note (original language) = 2'-methoxy
  modified_base 19..20: mod_base = OTHER; note; note (original language) = 3'-phosphorothioate
  modified_base 2: mod_base = OTHER; note; note (original language) = Guanosine-glycol nucleic acid
  modified_base 3..5: mod_base = OTHER; note; note (original language) = 2'-methoxy
  modified_base 7: mod_base = OTHER; note; note (original language) = 2'-methoxy
  modified_base 9..11: mod_base = OTHER; note; note (original language) = 2'-methoxy
  modified_base 13: mod_base = OTHER; note; note (original language) = 2'-methoxy
  modified_base 15: mod_base = OTHER; note; note (original language) = 2'-methoxy
  modified_base 17: mod_base = OTHER; note; note (original language) = 2'-methoxy
  modified_base 19..21: mod_base = OTHER; note; note (original language) = 2'-methoxy
  modified_base 6: mod_base = OTHER; note; note (original language) = 2'-deoxy-2'-fluoro
  modified_base 8: mod_base = OTHER; note; note (original language) = 2'-deoxy-2'-fluoro
  modified_base 12: mod_base = OTHER; note; note (original language) = 2'-deoxy-2'-fluoro
  modified_base 14: mod_base = OTHER; note; note (original language) = 2'-deoxy-2'-fluoro
  modified_base 18: mod_base = OTHER; note; note (original language) = 2'-deoxy-2'-fluoro
  modified_base 13: mod_base = OTHER; note; note (original language) = N=hypoxanthine
tggtgaagcgaantgcacagg

SEQ ID NO: 6 - RNA, 21 nt, synthetic construct
  source 1..21: mol_type = other RNA
  modified_base 1..2: mod_base = OTHER; note; note (original language) = 2'-deoxy-2'-fluoro
  modified_base 19..20: mod_base = OTHER; note; note (original language) = 2'-deoxy-2'-fluoro
  modified_base 1: mod_base = OTHER; note; note (original language) = 2'-methoxy
  modified_base 4..5: mod_base = OTHER; note; note (original language) = 2'-methoxy
  modified_base 7: mod_base = OTHER; note; note (original language) = 2'-methoxy
  modified_base 9..11: mod_base = OTHER; note; note (original language) = 2'-methoxy
  modified_base 13: mod_base = OTHER; note; note (original language) = 2'-methoxy
  modified_base 15: mod_base = OTHER; note; note (original language) = 2'-methoxy
  modified_base 17: mod_base = OTHER; note; note (original language) = 2'-methoxy
  modified_base 19..21: mod_base = OTHER; note; note (original language) = 2'-methoxy
  modified_base 2: mod_base = OTHER; note; note (original language) = 2'-deoxy-2'-fluoro
  modified_base 6: mod_base = OTHER; note; note (original language) = 2'-deoxy-2'-fluoro
  modified_base 8: mod_base = OTHER; note; note (original language) = 2'-deoxy-2'-fluoro
  modified_base 12: mod_base = OTHER; note; note (original language) = 2'-deoxy-2'-fluoro
  modified_base 14: mod_base = OTHER; note; note (original language) = 2'-deoxy-2'-fluoro
  modified_base 16: mod_base = OTHER; note; note (original language) = 2'-deoxy-2'-fluoro
  modified_base 18: mod_base = OTHER; note; note (original language) = 2'-deoxy-2'-fluoro
  modified_base 3: mod_base = OTHER; note; note (original language) = Guanosine-glycol nucleic acid
  modified_base 13: mod_base = OTHER; note; note (original language) = N=hypoxanthine
tggtgaagcgaantgcacagg

SEQ ID NO: 7 - RNA, 21 nt, synthetic construct
  source 1..21: mol_type = other RNA
  modified_base 1..2: mod_base = OTHER; note; note (original language) = 3'-phosphorothioate
  modified_base 19..20: mod_base = OTHER; note; note (original language) = 3'-phosphorothioate
  modified_base 1: mod_base = OTHER; note; note (original language) = 2'-methoxy
  modified_base 3: mod_base = OTHER; note; note (original language) = 2'-methoxy
  modified_base 5: mod_base = OTHER; note; note (original language) = 2'-methoxy
  modified_base 7: mod_base = OTHER; note; note (original language) = 2'-methoxy
  modified_base 9..11: mod_base = OTHER; note; note (original language) = 2'-methoxy
  modified_base 13: mod_base = OTHER; note; note (original language) = 2'-methoxy
  modified_base 15: mod_base = OTHER; note; note (original language) = 2'-methoxy
  modified_base 17: mod_base = OTHER; note; note (original language) = 2'-methoxy
  modified_base 19..21: mod_base = OTHER; note; note (original language) = 2'-methoxy
  modified_base 2: mod_base = OTHER; note; note (original language) = 2'-deoxy-2'-fluoro
  modified_base 6: mod_base = OTHER; note; note (original language) = 2'-deoxy-2'-fluoro
  modified_base 8: mod_base = OTHER; note; note (original language) = 2'-deoxy-2'-fluoro
  modified_base 12: mod_base = OTHER; note; note (original language) = 2'-deoxy-2'-fluoro
  modified_base 14: mod_base = OTHER; note; note (original language) = 2'-deoxy-2'-fluoro
  modified_base 16: mod_base = OTHER; note; note (original language) = 2'-deoxy-2'-fluoro
  modified_base 18: mod_base = OTHER; note; note (original language) = 2'-deoxy-2'-fluoro
  modified_base 4: mod_base = OTHER; note; note (original language) = Uridine-glycol nucleic acid
  modified_base 13: mod_base = OTHER; note; note (original language) = N=hypoxanthine
tggtgaagcgaantgcacagg

SEQ ID NO: 8 - RNA, 21 nt, synthetic construct
  source 1..21: mol_type = other RNA
  modified_base 1..2: mod_base = OTHER; note; note (original language) = 3'-phosphorothioate
  modified_base 19..20: mod_base = OTHER; note; note (original language) = 3'-phosphorothioate
  modified_base 1: mod_base = OTHER; note; note (original language) = 2'-methoxy
  modified_base 3..4: mod_base = OTHER; note; note (original language) = 2'-methoxy
  modified_base 7: mod_base = OTHER; note; note (original language) = 2'-methoxy
  modified_base 7..11: mod_base = OTHER; note; note (original language) = 2'-methoxy
  modified_base 13: mod_base = OTHER; note; note (original language) = 2'-methoxy
  modified_base 15: mod_base = OTHER; note; note (original language) = 2'-methoxy
  modified_base 17: mod_base = OTHER; note; note (original language) = 2'-methoxy
  modified_base 19..21: mod_base = OTHER; note; note (original language) = 2'-methoxy
  modified_base 2: mod_base = OTHER; note; note (original language) = 2'-deoxy-2'-fluoro
  modified_base 6: mod_base = OTHER; note; note (original language) = 2'-deoxy-2'-fluoro
  modified_base 8: mod_base = OTHER; note; note (original language) = 2'-deoxy-2'-fluoro
  modified_base 12: mod_base = OTHER; note; note (original language) = 2'-deoxy-2'-fluoro
  modified_base 14: mod_base = OTHER; note; note (original language) = 2'-deoxy-2'-fluoro
  modified_base 16: mod_base = OTHER; note; note (original language) = 2'-deoxy-2'-fluoro
  modified_base 18: mod_base = OTHER; note; note (original language) = 2'-deoxy-2'-fluoro
  modified_base 5: mod_base = OTHER; note; note (original language) = Guanosine-glycol nucleic acid
  modified_base 13: mod_base = OTHER; note; note (original language) = N=hypoxanthine
tggtgaagcgaantgcacagg

SEQ ID NO: 9 - RNA, 21 nt, synthetic construct
  source 1..21: mol_type = other RNA
  modified_base 1..2: mod_base = OTHER; note; note (original language) = 3'-phosphorothioate
  modified_base 19..20: mod_base = OTHER; note; note (original language) = 3'-phosphorothioate
  modified_base 1: mod_base = OTHER; note; note (original language) = 2'-methoxy
  modified_base 3..5: mod_base = OTHER; note; note (original language) = 2'-methoxy
  modified_base 7: mod_base = OTHER; note; note (original language) = 2'-methoxy
  modified_base 9..11: mod_base = OTHER; note; note (original language) = 2'-methoxy
  modified_base 13: mod_base = OTHER; note; note (original language) = 2'-methoxy
  modified_base 15: mod_base = OTHER; note; note (original language) = 2'-methoxy
  modified_base 17: mod_base = OTHER; note; note (original language) = 2'-methoxy
  modified_base 19..21: mod_base = OTHER; note; note (original language) = 2'-methoxy
  modified_base 2: mod_base = OTHER; note; note (original language) = 2'-deoxy-2'-fluoro
  modified_base 8: mod_base = OTHER; note; note (original language) = 2'-deoxy-2'-fluoro
  modified_base 12: mod_base = OTHER; note; note (original language) = 2'-deoxy-2'-fluoro
  modified_base 14: mod_base = OTHER; note; note (original language) = 2'-deoxy-2'-fluoro
  modified_base 16: mod_base = OTHER; note; note (original language) = 2'-deoxy-2'-fluoro
  modified_base 18: mod_base = OTHER; note; note (original language) = 2'-deoxy-2'-fluoro
  modified_base 6: mod_base = OTHER; note; note (original language) = adenosine-glycol nucleic acid
  modified_base 13: mod_base = OTHER; note; note (original language) = N=hypoxanthine
tggtgaagcgaantgcacagg

SEQ ID NO: 10 - RNA, 21 nt, synthetic construct
  source 1..21: mol_type = other RNA
  modified_base 1..2: mod_base = OTHER; note; note (original language) = 3'-phosphorothioate
  modified_base 19..20: mod_base = OTHER; note; note (original language) = 3'-phosphorothioate
  modified_base 1: mod_base = OTHER; note; note (original language) = 2'-methoxy
  modified_base 3..5: mod_base = OTHER; note; note (original language) = 2'-methoxy
  modified_base 9..11: mod_base = OTHER; note; note (original language) = 2'-methoxy
  modified_base 13: mod_base = OTHER; note; note (original language) = 2'-methoxy
  modified_base 15: mod_base = OTHER; note; note (original language) = 2'-methoxy
  modified_base 17: mod_base = OTHER; note; note (original language) = 2'-methoxy
  modified_base 19..21: mod_base = OTHER; note; note (original language) = 2'-methoxy
  modified_base 2: mod_base = OTHER; note; note (original language) = 2'-deoxy-2'-fluoro
  modified_base 2: mod_base = OTHER; note; note (original language) = 2'-deoxy-2'-fluoro
  modified_base 6: mod_base = OTHER; note; note (original language) = 2'-deoxy-2'-fluoro
  modified_base 12: mod_base = OTHER; note; note (original language) = 2'-deoxy-2'-fluoro
  modified_base 14: mod_base = OTHER; note; note (original language) = 2'-deoxy-2'-fluoro
  modified_base 16: mod_base = OTHER; note; note (original language) = 2'-deoxy-2'-fluoro
  modified_base 18: mod_base = OTHER; note; note (original language) = 2'-deoxy-2'-fluoro
  modified_base 7: mod_base = OTHER; note; note (original language) = adenosine-glycol nucleic acid
  modified_base 13: mod_base = OTHER; note; note (original language) = N=hypoxanthine
tggtgaagcgaantgcacagg

SEQ ID NO: 11 - RNA, 21 nt, synthetic construct
  source 1..21: mol_type = other RNA
  modified_base 1..2: mod_base = OTHER; note; note (original language) = 3'-phosphorothioate
  modified_base 19..20: mod_base = OTHER; note; note (original language) = 3'-phosphorothioate
  modified_base 1: mod_base = OTHER; note; note (original language) = 2'-methoxy
  modified_base 3..5: mod_base = OTHER; note; note (original language) = 2'-methoxy
  modified_base 7: mod_base = OTHER; note; note (original language) = 2'-methoxy
  modified_base 9..11: mod_base = OTHER; note; note (original language) = 2'-methoxy
  modified_base 13: mod_base = OTHER; note; note (original language) = 2'-methoxy
  modified_base 15: mod_base = OTHER; note; note (original language) = 2'-methoxy
  modified_base 17: mod_base = OTHER; note; note (original language) = 2'-methoxy
  modified_base 19..21: mod_base = OTHER; note; note (original language) = 2'-methoxy
  modified_base 2: mod_base = OTHER; note; note (original language) = 2'-deoxy-2'-fluoro
  modified_base 6: mod_base = OTHER; note; note (original language) = 2'-deoxy-2'-fluoro
  modified_base 12: mod_base = OTHER; note; note (original language) = 2'-deoxy-2'-fluoro
  modified_base 14: mod_base = OTHER; note; note (original language) = 2'-deoxy-2'-fluoro
  modified_base 16: mod_base = OTHER; note; note (original language) = 2'-deoxy-2'-fluoro
  modified_base 18: mod_base = OTHER; note; note (original language) = 2'-deoxy-2'-fluoro
  modified_base 8: mod_base = OTHER; note = Ggn; note (original language) = Guanosine-glycol nucleic acid
  modified_base 13: mod_base = OTHER; note; note (original language) = N=hypoxanthine
tggtgaagcgaantgcacagg

SEQ ID NO: 12 - RNA, 21 nt, synthetic construct
  source 1..21: mol_type = other RNA
  modified_base 19..20: mod_base = OTHER; note; note (original language) = 3'-phosphorothioate
  modified_base 1: mod_base = OTHER; note; note (original language) = 3'-phosphorothioate
  modified_base 1: mod_base = OTHER; note; note (original language) = 2'-methoxy
  modified_base 3..5: mod_base = OTHER; note; note (original language) = 2'-methoxy
  modified_base 7: mod_base = OTHER; note; note (original language) = 2'-methoxy
  modified_base 9..11: mod_base = OTHER; note; note (original language) = 2'-methoxy
  modified_base 13: mod_base = OTHER; note; note (original language) = 2'-methoxy
  modified_base 16: mod_base = OTHER; note; note (original language) = 2'-methoxy
  modified_base 17: mod_base = OTHER; note; note (original language) = 2'-methoxy
  modified_base 19..21: mod_base = OTHER; note; note (original language) = 2'-methoxy
  modified_base 6: mod_base = OTHER; note; note (original language) = 2'-deoxy-2'-fluoro
  modified_base 12: mod_base = OTHER; note; note (original language) = 2'-deoxy-2'-fluoro
  modified_base 14: mod_base = OTHER; note; note (original language) = 2'-deoxy-2'-fluoro
  modified_base 16: mod_base = OTHER; note; note (original language) = 2'-deoxy-2'-fluoro
  modified_base 18: mod_base = OTHER; note; note (original language) = 2'-deoxy-2'-fluoro
  modified_base 2: mod_base = OTHER; note; note (original language) = 2'-O-methoxyethyl
  modified_base 13: mod_base = OTHER; note; note (original language) = N=hypoxanthine
tggtgaagcgaantgcacagg

SEQ ID NO: 13 - RNA, 21 nt, synthetic construct
  source 1..21: mol_type = other RNA
  modified_base 1..2: mod_base = OTHER; note; note (original language) = 3'-phosphorothioate
  modified_base 19..20: mod_base = OTHER; note; note (original language) = 3'-phosphorothioate
  modified_base 1: mod_base = OTHER; note; note (original language) = 2'-methoxy
  modified_base 4..5: mod_base = OTHER; note; note (original language) = 2'-methoxy
  modified_base 7: mod_base = OTHER; note; note (original language) = 2'-methoxy
  modified_base 9..11: mod_base = OTHER; note; note (original language) = 2'-methoxy
  modified_base 13: mod_base = OTHER; note; note (original language) = 2'-methoxy
  modified_base 15: mod_base = OTHER; note; note (original language) = 2'-methoxy
  modified_base 17: mod_base = OTHER; note; note (original language) = 2'-methoxy
  modified_base 19..21: mod_base = OTHER; note; note (original language) = 2'-methoxy
  modified_base 2: mod_base = OTHER; note; note (original language) = 2'-deoxy-2'-fluoro
  modified_base 5: mod_base = OTHER; note; note (original language) = 2'-deoxy-2'-fluoro
  modified_base 8: mod_base = OTHER; note; note (original language) = 2'-deoxy-2'-fluoro
  modified_base 12: mod_base = OTHER; note; note (original language) = 2'-deoxy-2'-fluoro
  modified_base 14: mod_base = OTHER; note; note (original language) = 2'-deoxy-2'-fluoro
  modified_base 16: mod_base = OTHER; note; note (original language) = 2'-deoxy-2'-fluoro
  modified_base 18: mod_base = OTHER; note; note (original language) = 2'-deoxy-2'-fluoro
  modified_base 3: mod_base = OTHER; note; note (original language) = 2'-O-methoxyethyl
  modified_base 13: mod_base = OTHER; note; note (original language) = N=hypoxanthine
tggtgaagcgaantgcacagg

SEQ ID NO: 14 - RNA, 21 nt, synthetic construct
  source 1..21: mol_type = other RNA
  modified_base 1..2: mod_base = OTHER; note; note (original language) = 3'-phosphorothioate
  modified_base 19..20: mod_base = OTHER; note; note (original language) = 3'-phosphorothioate
  modified_base 4: mod_base = OTHER; note; note (original language) = 2'-O-methoxyethyl
  modified_base 1: mod_base = OTHER; note; note (original language) = 2'-methoxy
  modified_base 3: mod_base = OTHER; note; note (original language) = 2'-methoxy
  modified_base 7: mod_base = OTHER; note; note (original language) = 2'-methoxy
  modified_base 9..11: mod_base = OTHER; note; note (original language) = 2'-methoxy
  modified_base 13: mod_base = OTHER; note; note (original language) = 2'-methoxy
  modified_base 15: mod_base = OTHER; note; note (original language) = 2'-methoxy
  modified_base 17: mod_base = OTHER; note; note (original language) = 2'-methoxy
  modified_base 19..21: mod_base = OTHER; note; note (original language) = 2'-methoxy
  modified_base 2: mod_base = OTHER; note; note (original language) = 2'-deoxy-2'-fluoro
  modified_base 6: mod_base = OTHER; note; note (original language) = 2'-deoxy-2'-fluoro
  modified_base 8: mod_base = OTHER; note; note (original language) = 2'-deoxy-2'-fluoro
  modified_base 12: mod_base = OTHER; note; note (original language) = 2'-deoxy-2'-fluoro
  modified_base 14: mod_base = OTHER; note; note (original language) = 2'-deoxy-2'-fluoro
  modified_base 16: mod_base = OTHER; note; note (original language) = 2'-deoxy-2'-fluoro
  modified_base 18: mod_base = OTHER; note; note (original language) = 2'-deoxy-2'-fluoro
  modified_base 5: mod_base = OTHER; note; note (original language) = 2'-methoxy
  modified_base 13: mod_base = OTHER; note; note (original language) = N=hypoxanthine
  modified_base 13: mod_base = OTHER; note; note (original language) = N=hypoxanthine
tggtgaagcgaantgcacagg

SEQ ID NO: 15 - RNA, 21 nt, synthetic construct
  source 1..21: mol_type = other RNA
  modified_base 1..2: mod_base = OTHER; note; note (original language) = 3'-phosphorothioate
  modified_base 19..20: mod_base = OTHER; note; note (original language) = 3'-phosphorothioate
  modified_base 1: mod_base = OTHER; note; note (original language) = 2'-methoxy
  modified_base 3..4: mod_base = OTHER; note; note (original language) = 2'-methoxy
  modified_base 7: mod_base = OTHER; note; note (original language) = 2'-methoxy
  modified_base 9..11: mod_base = OTHER; note; note (original language) = 2'-methoxy
  modified_base 13: mod_base = OTHER; note; note (original language) = 2'-methoxy
  modified_base 13: mod_base = OTHER; note; note (original language) = 2'-methoxy
  modified_base 15: mod_base = OTHER; note; note (original language) = 2'-methoxy
  modified_base 17: mod_base = OTHER; note; note (original language) = 2'-methoxy
  modified_base 19..21: mod_base = OTHER; note; note (original language) = 2'-methoxy
  modified_base 2: mod_base = OTHER; note; note (original language) = 2'-deoxy-2'-fluoro
  modified_base 6: mod_base = OTHER; note; note (original language) = 2'-O-methoxyethyl
  modified_base 8: mod_base = OTHER; note; note (original language) = 2'-deoxy-2'-fluoro
  modified_base 12: mod_base = OTHER; note; note (original language) = 2'-deoxy-2'-fluoro
  modified_base 14: mod_base = OTHER; note; note (original language) = 2'-deoxy-2'-fluoro
  modified_base 16: mod_base = OTHER; note; note (original language) = 2'-deoxy-2'-fluoro
  modified_base 18: mod_base = OTHER; note; note (original language) = 2'-deoxy-2'-fluoro
  modified_base 5: mod_base = OTHER; note; note (original language) = 2'-O-methoxyethyl
  modified_base 13: mod_base = OTHER; note; note (original language) = N=hypoxanthine
tggtgaagcgaantgcacagg

SEQ ID NO: 16 - RNA, 21 nt, synthetic construct
  source 1..21: mol_type = other RNA
  modified_base 1..2: mod_base = OTHER; note; note (original language) = 3'-phosphorothioate
  modified_base 19..20: mod_base = OTHER; note; note (original language) = 3'-phosphorothioate
  modified_base 6: mod_base = OTHER; note; note (original language) = 2'-O-methoxyethyl
  modified_base 1: mod_base = OTHER; note; note (original language) = 2'-methoxy
  modified_base 3..5: mod_base = OTHER; note; note (original language) = 2'-methoxy
  modified_base 7: mod_base = OTHER; note; note (original language) = 2'-methoxy
  modified_base 9..11: mod_base = OTHER; note; note (original language) = 2'-methoxy
  modified_base 13: mod_base = OTHER; note; note (original language) = 2'-methoxy
  modified_base 15: mod_base = OTHER; note; note (original language) = 2'-methoxy
  modified_base 17: mod_base = OTHER; note; note (original language) = 2'-methoxy
  modified_base 19..21: mod_base = OTHER; note; note (original language) = 2'-methoxy
  modified_base 2: mod_base = OTHER; note; note (original language) = 2'-deoxy-2'-fluoro
  modified_base 8: mod_base = OTHER; note; note (original language) = 2'-deoxy-2'-fluoro
  modified_base 12: mod_base = OTHER; note; note (original language) = 2'-deoxy-2'-fluoro
  modified_base 14: mod_base = OTHER; note; note (original language) = 2'-deoxy-2'-fluoro
  modified_base 16: mod_base = OTHER; note; note (original language) = 2'-deoxy-2'-fluoro
  modified_base 18: mod_base = OTHER; note; note (original language) = 2'-deoxy-2'-fluoro
  modified_base 13: mod_base = OTHER; note; note (original language) = N=hypoxanthine
tggtgaagcgaantgcacagg

SEQ ID NO: 17 - RNA, 21 nt, synthetic construct
  source 1..21: mol_type = other RNA
  modified_base 1..2: mod_base = OTHER; note; note (original language) = 3'-phosphorothioate
  modified_base 19..20: mod_base = OTHER; note; note (original language) = 3'-phosphorothioate
  modified_base 2: mod_base = OTHER; note; note (original language) = 2'-deoxy-2'-fluoro
  modified_base 6: mod_base = OTHER; note; note (original language) = 2'-deoxy-2'-fluoro
  modified_base 8: mod_base = OTHER; note; note (original language) = 2'-deoxy-2'-fluoro
  modified_base 12: mod_base = OTHER; note; note (original language) = 2'-deoxy-2'-fluoro
  modified_base 14: mod_base = OTHER; note; note (original language) = 2'-deoxy-2'-fluoro
  modified_base 16: mod_base = OTHER; note; note (original language) = 2'-deoxy-2'-fluoro
  modified_base 18: mod_base = OTHER; note; note (original language) = 2'-deoxy-2'-fluoro
  modified_base 1: mod_base = OTHER; note; note (original language) = 2'-methoxy
  modified_base 3..5: mod_base = OTHER; note; note (original language) = 2'-methoxy
  modified_base 9..11: mod_base = OTHER; note; note (original language) = 2'-methoxy
  modified_base 13: mod_base = OTHER; note; note (original language) = 2'-methoxy
  modified_base 15: mod_base = OTHER; note; note (original language) = 2'-methoxy
  modified_base 17: mod_base = OTHER; note; note (original language) = 2'-methoxy
  modified_base 19..21: mod_base = OTHER; note; note (original language) = 2'-methoxy
  modified_base 7: mod_base = OTHER; note; note (original language) = 2'-O-methoxyethyl
  modified_base 13: mod_base = OTHER; note; note (original language) = N=hypoxanthine
tggtgaagcgaantgcacagg

SEQ ID NO: 18 - RNA, 21 nt, synthetic construct
  source 1..21: mol_type = other RNA
  modified_base 1..2: mod_base = OTHER; note; note (original language) = 3'-phosphorothioate
  modified_base 19..20: mod_base = OTHER; note; note (original language) = 3'-phosphorothioate
  modified_base 8: mod_base = OTHER; note; note (original language) = 2'-O-methoxyethyl
  modified_base 1: mod_base = OTHER; note; note (original language) = 2'-methoxy
  modified_base 3..5: mod_base = OTHER; note; note (original language) = 2'-methoxy
  modified_base 7: mod_base = OTHER; note; note (original language) = 2'-methoxy
  modified_base 9..11: mod_base = OTHER; note; note (original language) = 2'-methoxy
  modified_base 13: mod_base = OTHER; note; note (original language) = 2'-methoxy
  modified_base 15: mod_base = OTHER; note; note (original language) = 2'-methoxy
  modified_base 17: mod_base = OTHER; note; note (original language) = 2'-methoxy
  modified_base 19..21: mod_base = OTHER; note; note (original language) = 2'-methoxy
  modified_base 2: mod_base = OTHER; note; note (original language) = 2'-deoxy-2'-fluoro
  modified_base 6: mod_base = OTHER; note; note (original language) = 2'-deoxy-2'-fluoro
  modified_base 12: mod_base = OTHER; note; note (original language) = 2'-deoxy-2'-fluoro
  modified_base 14: mod_base = OTHER; note; note (original language) = 2'-deoxy-2'-fluoro
  modified_base 16: mod_base = OTHER; note; note (original language) = 2'-deoxy-2'-fluoro
  modified_base 18: mod_base = OTHER; note; note (original language) = 2'-deoxy-2'-fluoro
  modified_base 13: mod_base = OTHER; note; note (original language) = N=hypoxanthine
tggtgaagcgaantgcacagg

SEQ ID NO: 19 - RNA, 21 nt, synthetic construct
  source 1..21: mol_type = other RNA
  modified_base 1..2: mod_base = OTHER; note; note (original language) = 3'-phosphorothioate
  modified_base 19..20: mod_base = OTHER; note; note (original language) = 3'-phosphorothioate
  modified_base 2: mod_base = OTHER; note; note (original language) = 2'-deoxy-2'-fluoro
  modified_base 6: mod_base = OTHER; note; note (original language) = 2'-deoxy-2'-fluoro
  modified_base 8: mod_base = OTHER; note; note (original language) = 2'-deoxy-2'-fluoro
  modified_base 12: mod_base = OTHER; note; note (original language) = 2'-deoxy-2'-fluoro
  modified_base 14: mod_base = OTHER; note; note (original language) = 2'-deoxy-2'-fluoro
  modified_base 16: mod_base = OTHER; note; note (original language) = 2'-deoxy-2'-fluoro
  modified_base 18: mod_base = OTHER; note; note (original language) = 2'-deoxy-2'-fluoro
  modified_base 1: mod_base = OTHER; note; note (original language) = 2'-methoxy
  modified_base 3: mod_base = OTHER; note; note (original language) = 2'-methoxy
  modified_base 5: mod_base = OTHER; note; note (original language) = 2'-methoxy
  modified_base 7: mod_base = OTHER; note; note (original language) = 2'-methoxy
  modified_base 9..11: mod_base = OTHER; note; note (original language) = 2'-methoxy
  modified_base 13: mod_base = OTHER; note; note (original language) = 2'-methoxy
  modified_base 15: mod_base = OTHER; note; note (original language) = 2'-methoxy
  modified_base 17: mod_base = OTHER; note; note (original language) = 2'-methoxy
  modified_base 19..21: mod_base = OTHER; note; note (original language) = 2'-methoxy
  modified_base 4: mod_base = OTHER; note; note (original language) = N=N-(2,3-dihydroxypropyl)-3,5-bis(trifluoromethyl)benzamide
  modified_base 13: mod_base = OTHER; note; note (original language) = N=hypoxanthine
tggngaagcgaantgcacagg

SEQ ID NO: 20 - RNA, 21 nt, synthetic construct
  source 1..21: mol_type = other RNA
  modified_base 1..2: mod_base = OTHER; note; note (original language) = 3'-phosphorothioate
  modified_base 19..20: mod_base = OTHER; note; note (original language) = 3'-phosphorothioate
  modified_base 1: mod_base = OTHER; note; note (original language) = 2'-methoxy
  modified_base 3..4: mod_base = OTHER; note; note (original language) = 2'-methoxy
  modified_base 7: mod_base = OTHER; note; note (original language) = 2'-methoxy
  modified_base 9..11: mod_base = OTHER; note; note (original language) = 2'-methoxy
  modified_base 13: mod_base = OTHER; note; note (original language) = 2'-methoxy
  modified_base 15: mod_base = OTHER; note; note (original language) = 2'-methoxy
  modified_base 17: mod_base = OTHER; note; note (original language) = 2'-methoxy
  modified_base 19..21: mod_base = OTHER; note; note (original language) = 2'-methoxy
  modified_base 2: mod_base = OTHER; note; note (original language) = 2'-deoxy-2'-fluoro
  modified_base 6: mod_base = OTHER; note; note (original language) = 2'-deoxy-2'-fluoro
  modified_base 8: mod_base = OTHER; note; note (original language) = 2'-deoxy-2'-fluoro
  modified_base 12: mod_base = OTHER; note; note (original language) = 2'-deoxy-2'-fluoro
  modified_base 14: mod_base = OTHER; note; note (original language) = 2'-deoxy-2'-fluoro
  modified_base 16: mod_base = OTHER; note; note (original language) = 2'-deoxy-2'-fluoro
  modified_base 18: mod_base = OTHER; note; note (original language) = 2'-deoxy-2'-fluoro
  modified_base 5: mod_base = OTHER; note; note (original language) = N=N-(2,3-dihydroxypropyl)-3,5-bis(trifluoromethyl)benzamide
  modified_base 13: mod_base = OTHER; note; note (original language) = N=hypoxanthine
tggtnaagcgaantgcacagg

SEQ ID NO: 21 - RNA, 21 nt, synthetic construct
  source 1..21: mol_type = other RNA
  modified_base 1..2: mod_base = OTHER; note; note (original language) = 3'-phosphorothioate
  modified_base 19..20: mod_base = OTHER; note; note (original language) = 3'-phosphorothioate
  modified_base 2: mod_base = OTHER; note; note (original language) = 2'-deoxy-2'-fluoro
  modified_base 8: mod_base = OTHER; note; note (original language) = 2'-deoxy-2'-fluoro
  modified_base 12: mod_base = OTHER; note; note (original language) = 2'-deoxy-2'-fluoro
  modified_base 14: mod_base = OTHER; note; note (original language) = 2'-deoxy-2'-fluoro
  modified_base 16: mod_base = OTHER; note; note (original language) = 2'-deoxy-2'-fluoro
  modified_base 18: mod_base = OTHER; note; note (original language) = 2'-deoxy-2'-fluoro
  modified_base 1: mod_base = OTHER; note; note (original language) = 2'-methoxy
  modified_base 3..5: mod_base = OTHER; note; note (original language) = 2'-methoxy
  modified_base 7: mod_base = OTHER; note; note (original language) = 2'-methoxy
  modified_base 9..11: mod_base = OTHER; note; note (original language) = 2'-methoxy
  modified_base 13: mod_base = OTHER; note; note (original language) = 2'-methoxy
  modified_base 15: mod_base = OTHER; note; note (original language) = 2'-methoxy
  modified_base 17: mod_base = OTHER; note; note (original language) = 2'-methoxy
  modified_base 19..21: mod_base = OTHER; note; note (original language) = 2'-methoxy
  modified_base 6: mod_base = OTHER; note; note (original language) = N=N-(2,3-dihydroxypropyl)-3,5-bis(trifluoromethyl)benzamide
  modified_base 13: mod_base = OTHER; note; note (original language) = N=hypoxanthine
tggtgnagcgaantgcacagg

SEQ ID NO: 22 - RNA, 21 nt, synthetic construct
  source 1..21: mol_type = other RNA
  modified_base 1..2: mod_base = OTHER; note; note (original language) = 3'-phosphorothioate
  modified_base 19..20: mod_base = OTHER; note; note (original language) = 3'-phosphorothioate
  modified_base 1: mod_base = OTHER; note; note (original language) = 2'-methoxy
  modified_base 3..5: mod_base = OTHER; note; note (original language) = 2'-methoxy
  modified_base 9..11: mod_base = OTHER; note; note (original language) = 2'-methoxy
  modified_base 13: mod_base = OTHER; note; note (original language) = 2'-methoxy
  modified_base 15: mod_base = OTHER; note; note (original language) = 2'-methoxy
  modified_base 17: mod_base = OTHER; note; note (original language) = 2'-methoxy
  modified_base 19..21: mod_base = OTHER; note; note (original language) = 2'-methoxy
  modified_base 2: mod_base = OTHER; note; note (original language) = 2'-deoxy-2'-fluoro
  modified_base 6: mod_base = OTHER; note; note (original language) = 2'-deoxy-2'-fluoro
  modified_base 8: mod_base = OTHER; note; note (original language) = 2'-deoxy-2'-fluoro
  modified_base 12: mod_base = OTHER; note; note (original language) = 2'-deoxy-2'-fluoro
  modified_base 14: mod_base = OTHER; note; note (original language) = 2'-deoxy-2'-fluoro
  modified_base 16: mod_base = OTHER; note; note (original language) = 2'-deoxy-2'-fluoro
  modified_base 18: mod_base = OTHER; note; note (original language) = 2'-deoxy-2'-fluoro
  modified_base 7: mod_base = OTHER; note; note (original language) = N=N-(2,3-dihydroxypropyl)-3,5-bis(trifluoromethyl)benzamide
  modified_base 13: mod_base = OTHER; note; note (original language) = N=hypoxanthine
tggtgangcgaantgcacagg

SEQ ID NO: 23 - RNA, 21 nt, synthetic construct
  source 1..21: mol_type = other RNA
  modified_base 1..2: mod_base = OTHER; note; note (original language) = 3'-phosphorothioate
  modified_base 19..20: mod_base = OTHER; note; note (original language) = 3'-phosphorothioate
  modified_base 2: mod_base = OTHER; note; note (original language) = 2'-deoxy-2'-fluoro
  modified_base 6: mod_base = OTHER; note; note (original language) = 2'-deoxy-2'-fluoro
  modified_base 8: mod_base = OTHER; note; note (original language) = 2'-deoxy-2'-fluoro
  modified_base 12: mod_base = OTHER; note; note (original language) = 2'-deoxy-2'-fluoro
  modified_base 14: mod_base = OTHER; note; note (original language) = 2'-deoxy-2'-fluoro
  modified_base 16: mod_base = OTHER; note; note (original language) = 2'-deoxy-2'-fluoro
  modified_base 18: mod_base = OTHER; note; note (original language) = 2'-deoxy-2'-fluoro
  modified_base 1: mod_base = OTHER; note; note (original language) = 2'-methoxy
  modified_base 3: mod_base = OTHER; note; note (original language) = 2'-methoxy
  modified_base 5: mod_base = OTHER; note; note (original language) = 2'-methoxy
  modified_base 7: mod_base = OTHER; note; note (original language) = 2'-methoxy
  modified_base 9..11: mod_base = OTHER; note; note (original language) = 2'-methoxy
  modified_base 13: mod_base = OTHER; note; note (original language) = 2'-methoxy
  modified_base 15: mod_base = OTHER; note; note (original language) = 2'-methoxy
  modified_base 17: mod_base = OTHER; note; note (original language) = 2'-methoxy
  modified_base 19..21: mod_base = OTHER; note; note (original language) = 2'-methoxy
  modified_base 4: mod_base = OTHER; note; note (original language) = uridine-2' phosphate
  modified_base 13: mod_base = OTHER; note; note (original language) = N=hypoxanthine
tggtgaagcgaantgcacagg

SEQ ID NO: 24 - RNA, 21 nt, synthetic construct
  source 1..21: mol_type = other RNA
  modified_base 1..2: mod_base = OTHER; note; note (original language) = 3'-phosphorothioate
  modified_base 19..20: mod_base = OTHER; note; note (original language) = 3'-phosphorothioate
  modified_base 1: mod_base = OTHER; note; note (original language) = 2'-methoxy
  modified_base 3..4: mod_base = OTHER; note; note (original language) = 2'-methoxy
  modified_base 7: mod_base = OTHER; note; note (original language) = 2'-methoxy
  modified_base 9..11: mod_base = OTHER; note; note (original language) = 2'-methoxy
  modified_base 13: mod_base = OTHER; note; note (original language) = 2'-methoxy
  modified_base 15: mod_base = OTHER; note; note (original language) = 2'-methoxy
  modified_base 17: mod_base = OTHER; note; note (original language) = 2'-methoxy
  modified_base 19..21: mod_base = OTHER; note; note (original language) = 2'-methoxy
  modified_base 2: mod_base = OTHER; note; note (original language) = 2'-deoxy-2'-fluoro
  modified_base 6: mod_base = OTHER; note; note (original language) = 2'-deoxy-2'-fluoro
  modified_base 8: mod_base = OTHER; note; note (original language) = 2'-deoxy-2'-fluoro
  modified_base 16: mod_base = OTHER; note; note (original language) = 2'-deoxy-2'-fluoro
  modified_base 12: mod_base = OTHER; note; note (original language) = 2'-deoxy-2'-fluoro
  modified_base 14: mod_base = OTHER; note; note (original language) = 2'-deoxy-2'-fluoro
  modified_base 18: mod_base = OTHER; note; note (original language) = 2'-deoxy-2'-fluoro
  modified_base 5: mod_base = OTHER; note; note (original language) = uridine-2' phosphate
  modified_base 13: mod_base = OTHER; note; note (original language) = N=hypoxanthine
tggtgaagcgaantgcacagg

SEQ ID NO: 25 - RNA, 21 nt, synthetic construct
  source 1..21: mol_type = other RNA
  modified_base 1..2: mod_base = OTHER; note; note (original language) = 3'-phosphorothioate
  modified_base 19..20: mod_base = OTHER; note; note (original language) = 3'-phosphorothioate
  modified_base 2: mod_base = OTHER; note; note (original language) = 2'-deoxy-2'-fluoro
  modified_base 8: mod_base = OTHER; note; note (original language) = 2'-deoxy-2'-fluoro
  modified_base 12: mod_base = OTHER; note; note (original language) = 2'-deoxy-2'-fluoro
  modified_base 14: mod_base = OTHER; note; note (original language) = 2'-deoxy-2'-fluoro
  modified_base 16: mod_base = OTHER; note; note (original language) = 2'-deoxy-2'-fluoro
  modified_base 18: mod_base = OTHER; note; note (original language) = 2'-deoxy-2'-fluoro
  modified_base 1: mod_base = OTHER; note; note (original language) = 2'-methoxy
  modified_base 3..5: mod_base = OTHER; note; note (original language) = 2'-methoxy
  modified_base 7: mod_base = OTHER; note; note (original language) = 2'-methoxy
  modified_base 9..11: mod_base = OTHER; note; note (original language) = 2'-methoxy
  modified_base 13: mod_base = OTHER; note; note (original language) = 2'-methoxy
  modified_base 17: mod_base = OTHER; note; note (original language) = 2'-methoxy
  modified_base 15: mod_base = OTHER; note; note (original language) = 2'-methoxy
  modified_base 19..21: mod_base = OTHER; note; note (original language) = 2'-methoxy
  modified_base 6: mod_base = OTHER; note; note (original language) = adenosine-2' phosphate
  modified_base 13: mod_base = OTHER; note; note (original language) = N=hypoxanthine
tggtgaagcgaantgcacagg

SEQ ID NO: 26 - RNA, 21 nt, synthetic construct
  source 1..21: mol_type = other RNA
  modified_base 1..2: mod_base = OTHER; note; note (original language) = 3'-phosphorothioate
  modified_base 19..20: mod_base = OTHER; note; note (original language) = 3'-phosphorothioate
  modified_base 1: mod_base = OTHER; note; note (original language) = 2'-methoxy
  modified_base 3..5: mod_base = OTHER; note; note (original language) = 2'-methoxy
  modified_base 9..11: mod_base = OTHER; note; note (original language) = 2'-methoxy
  modified_base 13: mod_base = OTHER; note; note (original language) = 2'-methoxy
  modified_base 15: mod_base = OTHER; note; note (original language) = 2'-methoxy
  modified_base 17: mod_base = OTHER; note; note (original language) = 2'-methoxy
  modified_base 19..21: mod_base = OTHER; note; note (original language) = 2'-methoxy
  modified_base 2: mod_base = OTHER; note; note (original language) = 2'-deoxy-2'-fluoro
  modified_base 6: mod_base = OTHER; note; note (original language) = 2'-deoxy-2'-fluoro
  modified_base 8: mod_base = OTHER; note; note (original language) = 2'-deoxy-2'-fluoro
  modified_base 12: mod_base = OTHER; note; note (original language) = 2'-deoxy-2'-fluoro
  modified_base 14: mod_base = OTHER; note; note (original language) = 2'-deoxy-2'-fluoro
  modified_base 16: mod_base = OTHER; note; note (original language) = 2'-deoxy-2'-fluoro
  modified_base 18: mod_base = OTHER; note; note (original language) = 2'-deoxy-2'-fluoro
  modified_base 7: mod_base = OTHER; note; note (original language) = adenosine-2' phosphate
  modified_base 13: mod_base = OTHER; note; note (original language) = N=hypoxanthine
tggtgaagcgaantgcacagg

SEQ ID NO: 27 - RNA, 21 nt, synthetic construct
  source 1..21: mol_type = other RNA
  modified_base 1..2: mod_base = OTHER; note; note (original language) = 3'-phosphorothioate
  modified_base 19..20: mod_base = OTHER; note; note (original language) = 3'-phosphorothioate
  modified_base 2: mod_base = OTHER; note; note (original language) = 2'-deoxy-2'-fluoro
  modified_base 6: mod_base = OTHER; note; note (original language) = 2'-deoxy-2'-fluoro
  modified_base 12: mod_base = OTHER; note; note (original language) = 2'-deoxy-2'-fluoro
  modified_base 14: mod_base = OTHER; note; note (original language) = 2'-deoxy-2'-fluoro
  modified_base 16: mod_base = OTHER; note; note (original language) = 2'-deoxy-2'-fluoro
  modified_base 18: mod_base = OTHER; note; note (original language) = 2'-deoxy-2'-fluoro
  modified_base 1: mod_base = OTHER; note = N=APU001; note (original language) = N=5'-vinylphosphonate-2'-N-acetyl-uridine
  modified_base 3..5: mod_base = OTHER; note; note (original language) = 2'-methoxy
  modified_base 6: mod_base = OTHER; note; note (original language) = 2'-methoxy
  modified_base 8: mod_base = OTHER; note; note (original language) = 2'-methoxy
  modified_base 12: mod_base = OTHER; note; note (original language) = 2'-methoxy
  modified_base 14: mod_base = OTHER; note; note (original language) = 2'-methoxy
  modified_base 16: mod_base = OTHER; note; note (original language) = 2'-methoxy
  modified_base 18: mod_base = OTHER; note; note (original language) = 2'-methoxy
  modified_base 1: mod_base = OTHER; note; note (original language) = N=5'-vinylphosphonate-2'-N-acetyl-uridine
  modified_base 13: mod_base = OTHER; note; note (original language) = N=hypoxanthine
nggtgaagcgaantgcacagg

SEQ ID NO: 28 - RNA, 21 nt, synthetic construct
  source 1..21: mol_type = other RNA
  modified_base 1..2: mod_base = OTHER; note; note (original language) = 3'-phosphorothioate
  modified_base 19..20: mod_base = OTHER; note; note (original language) = 3'-phosphorothioate
  modified_base 3..4: mod_base = OTHER; note; note (original language) = 2'-methoxy
  modified_base 7: mod_base = OTHER; note; note (original language) = 2'-methoxy
  modified_base 9..11: mod_base = OTHER; note; note (original language) = 2'-methoxy
  modified_base 13: mod_base = OTHER; note; note (original language) = 2'-methoxy
  modified_base 15: mod_base = OTHER; note; note (original language) = 2'-methoxy
  modified_base 17: mod_base = OTHER; note; note (original language) = 2'-methoxy
  modified_base 19..21: mod_base = OTHER; note; note (original language) = 2'-methoxy
  modified_base 2: mod_base = OTHER; note; note (original language) = 2'-deoxy-2'-fluoro
  modified_base 6: mod_base = OTHER; note; note (original language) = 2'-deoxy-2'-fluoro
  modified_base 6: mod_base = OTHER; note; note (original language) = 2'-deoxy-2'-fluoro
  modified_base 8: mod_base = OTHER; note; note (original language) = 2'-deoxy-2'-fluoro
  modified_base 12: mod_base = OTHER; note; note (original language) = 2'-deoxy-2'-fluoro
  modified_base 14: mod_base = OTHER; note; note (original language) = 2'-deoxy-2'-fluoro
  modified_base 16: mod_base = OTHER; note; note (original language) = 2'-deoxy-2'-fluoro
  modified_base 18: mod_base = OTHER; note; note (original language) = 2'-deoxy-2'-fluoro
  modified_base 5: mod_base = OTHER; note; note (original language) = Guanosine-glycol nucleic acid
  modified_base 1: mod_base = OTHER; note; note (original language) = N=5'-vinylphosphonate-2'-N-acetyl-uridine
  modified_base 13: mod_base = OTHER; note; note (original language) = N=hypoxanthine
nggtgaagcgaantgcacagg

SEQ ID NO: 29 - RNA, 21 nt, synthetic construct
  source 1..21: mol_type = other RNA
  modified_base 1..2: mod_base = OTHER; note; note (original language) = 3'-phosphorothioate
  modified_base 19..20: mod_base = OTHER; note; note (original language) = 3'-phosphorothioate
  modified_base 2: mod_base = OTHER; note; note (original language) = 2'-deoxy-2'-fluoro
  modified_base 6: mod_base = OTHER; note; note (original language) = 2'-deoxy-2'-fluoro
  modified_base 12: mod_base = OTHER; note; note (original language) = 2'-deoxy-2'-fluoro
  modified_base 14: mod_base = OTHER; note; note (original language) = 2'-deoxy-2'-fluoro
  modified_base 16: mod_base = OTHER; note; note (original language) = 2'-deoxy-2'-fluoro
  modified_base 18: mod_base = OTHER; note; note (original language) = 2'-deoxy-2'-fluoro
  modified_base 3..5: mod_base = OTHER; note; note (original language) = 2'-methoxy
  modified_base 9..11: mod_base = OTHER; note; note (original language) = 2'-methoxy
  modified_base 13: mod_base = OTHER; note; note (original language) = 2'-methoxy
  modified_base 15: mod_base = OTHER; note; note (original language) = 2'-methoxy
  modified_base 17: mod_base = OTHER; note; note (original language) = 2'-methoxy
  modified_base 19..21: mod_base = OTHER; note; note (original language) = 2'-methoxy
  modified_base 7: mod_base = OTHER; note; note (original language) = adenosine-glycol nucleic acid
  modified_base 1: mod_base = OTHER; note; note (original language) = N=5'-vinylphosphonate-2'-N-acetyl-uridine
  modified_base 13: mod_base = OTHER; note; note (original language) = N=hypoxanthine
nggtgaagcgaantgcacagg

SEQ ID NO: 30 - RNA, 21 nt, synthetic construct
  source 1..21: mol_type = other RNA
  modified_base 1..2: mod_base = OTHER; note; note (original language) = 3'-phosphorothioate
  modified_base 19..20: mod_base = OTHER; note; note (original language) = 3'-phosphorothioate
  modified_base 2: mod_base = OTHER; note; note (original language) = 2'-deoxy-2'-fluoro
  modified_base 6: mod_base = OTHER; note; note (original language) = 2'-deoxy-2'-fluoro
  modified_base 8: mod_base = OTHER; note; note (original language) = 2'-deoxy-2'-fluoro
  modified_base 12: mod_base = OTHER; note; note (original language) = 2'-deoxy-2'-fluoro
  modified_base 14: mod_base = OTHER; note; note (original language) = 2'-deoxy-2'-fluoro
  modified_base 16: mod_base = OTHER; note; note (original language) = 2'-deoxy-2'-fluoro
  modified_base 18: mod_base = OTHER; note; note (original language) = 2'-deoxy-2'-fluoro
  modified_base 3..4: mod_base = OTHER; note; note (original language) = 2'-methoxy
  modified_base 7: mod_base = OTHER; note; note (original language) = 2'-methoxy
  modified_base 9..11: mod_base = OTHER; note; note (original language) = 2'-methoxy
  modified_base 13: mod_base = OTHER; note; note (original language) = 2'-methoxy
  modified_base 15: mod_base = OTHER; note; note (original language) = 2'-methoxy
  modified_base 17: mod_base = OTHER; note; note (original language) = 2'-methoxy
  modified_base 19..21: mod_base = OTHER; note; note (original language) = 2'-methoxy
  modified_base 1: mod_base = OTHER; note; note (original language) = N=5'-vinylphosphonate-2'-N-acetyl-uridine
  modified_base 5: mod_base = OTHER; note; note (original language) = N=N-(2,3-dihydroxypropyl)-3,5-bis(trifluoromethyl)benzamide
  modified_base 13: mod_base = OTHER; note; note (original language) = N=hypoxanthine
nggtnaagcgaantgcacagg

SEQ ID NO: 31 - RNA, 21 nt, synthetic construct
  source 1..21: mol_type = other RNA
  modified_base 1..2: mod_base = OTHER; note; note (original language) = 3'-phosphorothioate
  modified_base 19..20: mod_base = OTHER; note; note (original language) = 3'-phosphorothioate
  modified_base 3..5: mod_base = OTHER; note; note (original language) = 2'-methoxy
  modified_base 9..11: mod_base = OTHER; note; note (original language) = 2'-methoxy
  modified_base 13: mod_base = OTHER; note; note (original language) = 2'-methoxy
  modified_base 15: mod_base = OTHER; note; note (original language) = 2'-methoxy
  modified_base 17: mod_base = OTHER; note; note (original language) = 2'-methoxy
  modified_base 19..21: mod_base = OTHER; note; note (original language) = 2'-methoxy
  modified_base 2: mod_base = OTHER; note; note (original language) = 2'-deoxy-2'-fluoro
  modified_base 6: mod_base = OTHER; note; note (original language) = 2'-deoxy-2'-fluoro
  modified_base 8: mod_base = OTHER; note; note (original language) = 2'-deoxy-2'-fluoro
  modified_base 12: mod_base = OTHER; note; note (original language) = 2'-deoxy-2'-fluoro
  modified_base 14: mod_base = OTHER; note; note (original language) = 2'-deoxy-2'-fluoro
  modified_base 16: mod_base = OTHER; note; note (original language) = 2'-deoxy-2'-fluoro
  modified_base 18: mod_base = OTHER; note; note (original language) = 2'-deoxy-2'-fluoro
  modified_base 7: mod_base = OTHER; note; note (original language) = N=N-(2,3-dihydroxypropyl)-3,5-bis(trifluoromethyl)benzamide
  modified_base 1: mod_base = OTHER; note; note (original language) = 5'-vinylphosphonate-2'-N-acetyl-uridine
  modified_base 7: mod_base = OTHER; note; note (original language) = N=N-(2,3-dihydroxypropyl)-3,5-bis(trifluoromethyl)benzamide
  modified_base 13: mod_base = OTHER; note; note (original language) = N=hypoxanthine
nggtgangcgaantgcacagg

SEQ ID NO: 32 - RNA, 21 nt, synthetic construct
  source 1..21: mol_type = other RNA
  modified_base 1..2: mod_base = OTHER; note; note (original language) = 3'-phosphorothioate
  modified_base 19..20: mod_base = OTHER; note; note (original language) = 3'-phosphorothioate
  modified_base 3..5: mod_base = OTHER; note; note (original language) = 2'-methoxy
  modified_base 9..11: mod_base = OTHER; note; note (original language) = 2'-methoxy
  modified_base 13: mod_base = OTHER; note; note (original language) = 2'-methoxy
  modified_base 15: mod_base = OTHER; note; note (original language) = 2'-methoxy
  modified_base 17: mod_base = OTHER; note; note (original language) = 2'-methoxy
  modified_base 19..21: mod_base = OTHER; note; note (original language) = 2'-methoxy
  modified_base 2: mod_base = OTHER; note; note (original language) = 2'-deoxy-2'-fluoro
  modified_base 6: mod_base = OTHER; note; note (original language) = 2'-deoxy-2'-fluoro
  modified_base 8: mod_base = OTHER; note; note (original language) = 2'-deoxy-2'-fluoro
  modified_base 12: mod_base = OTHER; note; note (original language) = 2'-deoxy-2'-fluoro
  modified_base 14: mod_base = OTHER; note; note (original language) = 2'-deoxy-2'-fluoro
  modified_base 16: mod_base = OTHER; note; note (original language) = 2'-deoxy-2'-fluoro
  modified_base 18: mod_base = OTHER; note; note (original language) = 2'-deoxy-2'-fluoro
  modified_base 1: mod_base = OTHER; note; note (original language) = N=5'-vinylphosphonate-2'-N-acetyl-uridine
  modified_base 7: mod_base = OTHER; note; note (original language) = adenosine-2' phosphate
  modified_base 13: mod_base = OTHER; note; note (original language) = N=hypoxanthine
nggtgaagcgaantgcacagg

SEQ ID NO: 33 - RNA, 21 nt, synthetic construct
  source 1..21: mol_type = other RNA
  modified_base 1..2: mod_base = OTHER; note; note (original language) = 3'-phosphorothioate
  modified_base 19..20: mod_base = OTHER; note; note (original language) = 3'-phosphorothioate
  modified_base 1: mod_base = OTHER; note; note (original language) = 2'-methoxy
  modified_base 3..5: mod_base = OTHER; note; note (original language) = 2'-methoxy
  modified_base 7..13: mod_base = OTHER; note; note (original language) = 2'-methoxy
  modified_base 15: mod_base = OTHER; note; note (original language) = 2'-methoxy
  modified_base 17..21: mod_base = OTHER; note; note (original language) = 2'-methoxy
  modified_base 2: mod_base = OTHER; note; note (original language) = 2'-deoxy-2'-fluoro
  modified_base 6: mod_base = OTHER; note; note (original language) = 2'-deoxy-2'-fluoro
  modified_base 14: mod_base = OTHER; note; note (original language) = 2'-deoxy-2'-fluoro
  modified_base 16: mod_base = OTHER; note; note (original language) = 2'-deoxy-2'-fluoro
  modified_base 1: mod_base = OTHER; note; note (original language) = 5'-vinylphosphonate
  modified_base 13: mod_base = OTHER; note; note (original language) = N=hypoxanthine
tggtgaagcgaantgcacagg

SEQ ID NO: 34 - RNA, 21 nt, synthetic construct
  source 1..21: mol_type = other RNA
  modified_base 1..2: mod_base = OTHER; note; note (original language) = 3'-phosphorothioate
  modified_base 19..20: mod_base = OTHER; note; note (original language) = 3'-phosphorothioate
  modified_base 2: mod_base = OTHER; note; note (original language) = 2'-deoxy-2'-fluoro
  modified_base 6: mod_base = OTHER; note; note (original language) = 2'-deoxy-2'-fluoro
  modified_base 8: mod_base = OTHER; note; note (original language) = 2'-deoxy-2'-fluoro
  modified_base 12: mod_base = OTHER; note; note (original language) = 2'-deoxy-2'-fluoro
  modified_base 14: mod_base = OTHER; note; note (original language) = 2'-deoxy-2'-fluoro
  modified_base 16: mod_base = OTHER; note; note (original language) = 2'-deoxy-2'-fluoro
  modified_base 18: mod_base = OTHER; note; note (original language) = 2'-deoxy-2'-fluoro
  modified_base 1: mod_base = OTHER; note; note (original language) = 2'-methoxy
  modified_base 3..4: mod_base = OTHER; note; note (original language) = 2'-methoxy
  modified_base 7: mod_base = OTHER; note; note (original language) = 2'-methoxy
  modified_base 9..11: mod_base = OTHER; note; note (original language) = 2'-methoxy
  modified_base 13: mod_base = OTHER; note; note (original language) = 2'-methoxy
  modified_base 15: mod_base = OTHER; note; note (original language) = 2'-methoxy
  modified_base 17: mod_base = OTHER; note; note (original language) = 2'-methoxy
  modified_base 19..21: mod_base = OTHER; note; note (original language) = 2'-methoxy
  modified_base 5: mod_base = OTHER; note; note (original language) = Guanosine-glycol nucleic acid
  modified_base 1: mod_base = OTHER; note; note (original language) = 5'-vinylphosphonate
  modified_base 13: mod_base = OTHER; note; note (original language) = N=hypoxanthine
tggtgaagcgaantgcacagg

SEQ ID NO: 35 - RNA, 21 nt, synthetic construct
  source 1..21: mol_type = other RNA
  modified_base 1..2: mod_base = OTHER; note; note (original language) = 3'-phosphorothioate
  modified_base 19..20: mod_base = OTHER; note; note (original language) = 3'-phosphorothioate
  modified_base 1: mod_base = OTHER; note; note (original language) = 2'-methoxy
  modified_base 3..5: mod_base = OTHER; note; note (original language) = 2'-methoxy
  modified_base 9..11: mod_base = OTHER; note; note (original language) = 2'-methoxy
  modified_base 13: mod_base = OTHER; note; note (original language) = 2'-methoxy
  modified_base 15: mod_base = OTHER; note; note (original language) = 2'-methoxy
  modified_base 17: mod_base = OTHER; note; note (original language) = 2'-methoxy
  modified_base 19..21: mod_base = OTHER; note; note (original language) = 2'-methoxy
  modified_base 2: mod_base = OTHER; note; note (original language) = 2'-deoxy-2'-fluoro
  modified_base 6: mod_base = OTHER; note; note (original language) = 2'-deoxy-2'-fluoro
  modified_base 8: mod_base = OTHER; note; note (original language) = 2'-deoxy-2'-fluoro
  modified_base 12: mod_base = OTHER; note; note (original language) = 2'-deoxy-2'-fluoro
  modified_base 14: mod_base = OTHER; note; note (original language) = 2'-deoxy-2'-fluoro
  modified_base 16: mod_base = OTHER; note; note (original language) = 2'-deoxy-2'-fluoro
  modified_base 18: mod_base = OTHER; note; note (original language) = 2'-deoxy-2'-fluoro
  modified_base 1: mod_base = OTHER; note; note (original language) = 5'-vinylphosphonate
  modified_base 7: mod_base = OTHER; note; note (original language) = adenosine-2' phosphate
  modified_base 15: mod_base = OTHER; note; note (original language) = N=hypoxanthine
tggtgaagcgaantgcacagg

SEQ ID NO: 36 - RNA, 19 nt, synthetic construct
  source 1..19: mol_type = other RNA
  modified_base 1..2: mod_base = OTHER; note; note (original language) = 3'-phosphorothioate
  modified_base 1..2: mod_base = OTHER; note; note (original language) = 3'-phosphorothioate
  modified_base 1..6: mod_base = OTHER; note; note (original language) = 2'-methoxy
  modified_base 8: mod_base = OTHER; note; note (original language) = 2'-methoxy
  modified_base 11..19: mod_base = OTHER; note; note (original language) = 2'-methoxy
  modified_base 7: mod_base = OTHER; note; note (original language) = 2'-deoxy-2'-fluoro
  modified_base 9..10: mod_base = OTHER; note; note (original language) = 2'-deoxy-2'-fluoro
tgtgcactccgcttcacca

SEQ ID NO: 37 - RNA, 19 nt, synthetic construct
  source 1..19: mol_type = other RNA
  modified_base 1..2: mod_base = OTHER; note; note (original language) = 3'-phosphorothioate
  modified_base 1..6: mod_base = OTHER; note; note (original language) = 2'-methoxy
  modified_base 10..19: mod_base = OTHER; note; note (original language) = 2'-methoxy
  modified_base 7..9: mod_base = OTHER; note; note (original language) = 2'-deoxy-2'-fluoro
ccttgaggcatacttcaaa

SEQ ID NO: 38 - RNA, 19 nt, synthetic construct
  source 1..19: mol_type = other RNA
  modified_base 1..2: mod_base = OTHER; note; note (original language) = 3'-phosphorothioate
  modified_base 7..9: mod_base = OTHER; note; note (original language) = 2'-deoxy-2'-fluoro
  modified_base 1..6: mod_base = OTHER; note; note (original language) = 2'-methoxy
  modified_base 10..19: mod_base = OTHER; note; note (original language) = 2'-methoxy
tgtgcactccgcttcacca

SEQ ID NO: 39 - RNA, 21 nt, synthetic construct
  source 1..21: mol_type = other RNA
  modified_base 1..2: mod_base = OTHER; note; note (original language) = 3'-phosphorothioate
  modified_base 19..20: mod_base = OTHER; note; note (original language) = 3'-phosphorothioate
  modified_base 1: mod_base = OTHER; note; note (original language) = 2'-methoxy
  modified_base 3..5: mod_base = OTHER; note; note (original language) = 2'-methoxy
  modified_base 7..13: mod_base = OTHER; note; note (original language) = 2'-methoxy
  modified_base 15: mod_base = OTHER; note; note (original language) = 2'-methoxy
  modified_base 17..21: mod_base = OTHER; note; note (original language) = 2'-methoxy
  modified_base 2: mod_base = OTHER; note; note (original language) = 2'-deoxy-2'-fluoro
  modified_base 6: mod_base = OTHER; note; note (original language) = 2'-deoxy-2'-fluoro
  modified_base 14: mod_base = OTHER; note; note (original language) = 2'-deoxy-2'-fluoro
  modified_base 16: mod_base = OTHER; note; note (original language) = 2'-deoxy-2'-fluoro
  modified_base 1: mod_base = OTHER; note; note (original language) = 5'-vinylphosphonate
tttgaagtatgcctcaaggtt

SEQ ID NO: 40 - RNA, 19 nt, synthetic construct
  source 1..19: mol_type = other RNA
  modified_base 1..2: mod_base = OTHER; note; note (original language) = 3'-phosphorothioate
  modified_base 1..6: mod_base = OTHER; note; note (original language) = 2'-methoxy
  modified_base 8: mod_base = OTHER; note; note (original language) = 2'-methoxy
  modified_base 12..19: mod_base = OTHER; note; note (original language) = 2'-methoxy
  modified_base 7: mod_base = OTHER; note; note (original language) = 2'-deoxy-2'-fluoro
  modified_base 9..11: mod_base = OTHER; note; note (original language) = 2'-deoxy-2'-fluoro
gccggaccgtgtgcacttc

SEQ ID NO: 41 - RNA, 19 nt, synthetic construct
  source 1..19: mol_type = other RNA
  modified_base 1..2: mod_base = OTHER; note; note (original language) = 3'-phosphorothioate
  modified_base 1..6: mod_base = OTHER; note; note (original language) = 2'-methoxy
  modified_base 8: mod_base = OTHER; note; note (original language) = 2'-methoxy
  modified_base 12..19: mod_base = OTHER; note; note (original language) = 2'-methoxy
  modified_base 7: mod_base = OTHER; note; note (original language) = 2'-deoxy-2'-fluoro
  modified_base 9..11: mod_base = OTHER; note; note (original language) = 2'-deoxy-2'-fluoro
tgtgcacttcgcttcacca

SEQ ID NO: 42 - RNA, 19 nt, synthetic construct
  source 1..19: mol_type = other RNA
  modified_base 1..2: mod_base = OTHER; note; note (original language) = 3'-phosphorothioate
  modified_base 7: mod_base = OTHER; note; note (original language) = 2'-deoxy-2'-fluoro
  modified_base 9..11: mod_base = OTHER; note; note (original language) = 2'-deoxy-2'-fluoro
  modified_base 1..6: mod_base = OTHER; note; note (original language) = 2'-methoxy
  modified_base 8: mod_base = OTHER; note; note (original language) = 2'-methoxy
  modified_base 12..19: mod_base = OTHER; note; note (original language) = 2'-methoxy
ccgtgtgcacttcgcttca

SEQ ID NO: 43 - RNA, 19 nt, synthetic construct
  source 1..19: mol_type = other RNA
  modified_base 1..2: mod_base = OTHER; note; note (original language) = 3'-phosphorothioate
  modified_base 1..6: mod_base = OTHER; note; note (original language) = 2'-methoxy
  modified_base 8: mod_base = OTHER; note; note (original language) = 2'-methoxy
  modified_base 12..19: mod_base = OTHER; note; note (original language) = 2'-methoxy
  modified_base 7: mod_base = OTHER; note; note (original language) = 2'-deoxy-2'-fluoro
  modified_base 9..11: mod_base = OTHER; note; note (original language) = 2'-deoxy-2'-fluoro
gaccgtgtgcacttcgcta

SEQ ID NO: 44 - RNA, 19 nt, synthetic construct
  source 1..19: mol_type = other RNA
  modified_base 1..2: mod_base = OTHER; note; note (original language) = 3'-phosphorothioate
  modified_base 7: mod_base = OTHER; note; note (original language) = 2'-deoxy-2'-fluoro
  modified_base 9: mod_base = OTHER; note; note (original language) = 2'-deoxy-2'-fluoro
  modified_base 11: mod_base = OTHER; note; note (original language) = 2'-deoxy-2'-fluoro
  modified_base 1..6: mod_base = OTHER; note; note (original language) = 2'-methoxy
  modified_base 8: mod_base = OTHER; note; note (original language) = 2'-methoxy
  modified_base 10: mod_base = OTHER; note; note (original language) = 2'-methoxy
  modified_base 12..19: mod_base = OTHER; note; note (original language) = 2'-methoxy
gaccgtgtgcacttcgcta

SEQ ID NO: 45 - RNA, 19 nt, synthetic construct
  source 1..19: mol_type = other RNA
  modified_base 1..2: mod_base = OTHER; note; note (original language) = 3'-phosphorothioate
  modified_base 1..6: mod_base = OTHER; note; note (original language) = 2'-methoxy
  modified_base 8: mod_base = OTHER; note; note (original language) = 2'-methoxy
  modified_base 11..19: mod_base = OTHER; note; note (original language) = 2'-methoxy
  modified_base 7: mod_base = OTHER; note; note (original language) = 2'-deoxy-2'-fluoro
  modified_base 9..10: mod_base = OTHER; note; note (original language) = 2'-deoxy-2'-fluoro
gaccgtgtgcacttcgcta

SEQ ID NO: 46 - RNA, 19 nt, synthetic construct
  source 1..19: mol_type = other RNA
  modified_base 1..2: mod_base = OTHER; note; note (original language) = 3'-phosphorothioate
  modified_base 7: mod_base = OTHER; note; note (original language) = 2'-deoxy-2'-fluoro
  modified_base 10..11: mod_base = OTHER; note; note (original language) = 2'-deoxy-2'-fluoro
  modified_base 1..6: mod_base = OTHER; note; note (original language) = 2'-methoxy
  modified_base 8..9: mod_base = OTHER; note; note (original language) = 2'-methoxy
  modified_base 12..19: mod_base = OTHER; note; note (original language) = 2'-methoxy
gaccgtgtgcacttcgcta

SEQ ID NO: 47 - RNA, 21 nt, synthetic construct
  source 1..21: mol_type = other RNA
  modified_base 1..2: mod_base = OTHER; note; note (original language) = 3'-phosphorothioate
  modified_base 19..20: mod_base = OTHER; note; note (original language) = 3'-phosphorothioate
  modified_base 1: mod_base = OTHER; note; note (original language) = 2'-methoxy
  modified_base 3..5: mod_base = OTHER; note; note (original language) = 2'-methoxy
  modified_base 7: mod_base = OTHER; note; note (original language) = 2'-methoxy
  modified_base 9..11: mod_base = OTHER; note; note (original language) = 2'-methoxy
  modified_base 13: mod_base = OTHER; note; note (original language) = 2'-methoxy
  modified_base 15: mod_base = OTHER; note; note (original language) = 2'-methoxy
  modified_base 17: mod_base = OTHER; note; note (original language) = 2'-methoxy
  modified_base 19..21: mod_base = OTHER; note; note (original language) = 2'-methoxy
  modified_base 2: mod_base = OTHER; note; note (original language) = 2'-deoxy-2'-fluoro
  modified_base 6: mod_base = OTHER; note; note (original language) = 2'-deoxy-2'-fluoro
  modified_base 8: mod_base = OTHER; note; note (original language) = 2'-deoxy-2'-fluoro
  modified_base 12: mod_base = OTHER; note; note (original language) = 2'-deoxy-2'-fluoro
  modified_base 14: mod_base = OTHER; note; note (original language) = 2'-deoxy-2'-fluoro
  modified_base 16: mod_base = OTHER; note; note (original language) = 2'-deoxy-2'-fluoro
  modified_base 18: mod_base = OTHER; note; note (original language) = 2'-deoxy-2'-fluoro
gaagtgcacacggtccggcag

SEQ ID NO: 48 - RNA, 21 nt, synthetic construct
  source 1..21: mol_type = other RNA
  modified_base 1..2: mod_base = OTHER; note; note (original language) = 3'-phosphorothioate
  modified_base 19..20: mod_base = OTHER; note; note (original language) = 3'-phosphorothioate
  modified_base 1: mod_base = OTHER; note; note (original language) = 2'-methoxy
  modified_base 3..5: mod_base = OTHER; note; note (original language) = 2'-methoxy
  modified_base 7: mod_base = OTHER; note; note (original language) = 2'-methoxy
  modified_base 9..11: mod_base = OTHER; note; note (original language) = 2'-methoxy
  modified_base 13: mod_base = OTHER; note; note (original language) = 2'-methoxy
  modified_base 15: mod_base = OTHER; note; note (original language) = 2'-methoxy
  modified_base 17: mod_base = OTHER; note; note (original language) = 2'-methoxy
  modified_base 19..21: mod_base = OTHER; note; note (original language) = 2'-methoxy
  modified_base 2: mod_base = OTHER; note; note (original language) = 2'-deoxy-2'-fluoro
  modified_base 6: mod_base = OTHER; note; note (original language) = 2'-deoxy-2'-fluoro
  modified_base 8: mod_base = OTHER; note; note (original language) = 2'-deoxy-2'-fluoro
  modified_base 12: mod_base = OTHER; note; note (original language) = 2'-deoxy-2'-fluoro
  modified_base 14: mod_base = OTHER; note; note (original language) = 2'-deoxy-2'-fluoro
  modified_base 16: mod_base = OTHER; note; note (original language) = 2'-deoxy-2'-fluoro
  modified_base 18: mod_base = OTHER; note; note (original language) = 2'-deoxy-2'-fluoro
tggtgaagcgaagtgcacagg

SEQ ID NO: 49 - RNA, 21 nt, synthetic construct
  source 1..21: mol_type = other RNA
  modified_base 1..2: mod_base = OTHER; note; note (original language) = 3'-phosphorothioate
  modified_base 19..20: mod_base = OTHER; note; note (original language) = 3'-phosphorothioate
  modified_base 1: mod_base = OTHER; note; note (original language) = 2'-methoxy
  modified_base 3..5: mod_base = OTHER; note; note (original language) = 2'-methoxy
  modified_base 7: mod_base = OTHER; note; note (original language) = 2'-methoxy
  modified_base 9..11: mod_base = OTHER; note; note (original language) = 2'-methoxy
  modified_base 13: mod_base = OTHER; note; note (original language) = 2'-methoxy
  modified_base 15: mod_base = OTHER; note; note (original language) = 2'-methoxy
  modified_base 17: mod_base = OTHER; note; note (original language) = 2'-methoxy
  modified_base 19..21: mod_base = OTHER; note; note (original language) = 2'-methoxy
  modified_base 2: mod_base = OTHER; note; note (original language) = 2'-deoxy-2'-fluoro
  modified_base 6: mod_base = OTHER; note; note (original language) = 2'-deoxy-2'-fluoro
  modified_base 8: mod_base = OTHER; note; note (original language) = 2'-deoxy-2'-fluoro
  modified_base 12: mod_base = OTHER; note; note (original language) = 2'-deoxy-2'-fluoro
  modified_base 14: mod_base = OTHER; note; note (original language) = 2'-deoxy-2'-fluoro
  modified_base 16: mod_base = OTHER; note; note (original language) = 2'-deoxy-2'-fluoro
  modified_base 18: mod_base = OTHER; note; note (original language) = 2'-deoxy-2'-fluoro
tgaagcgaagtgcacacggtc

SEQ ID NO: 50 - RNA, 21 nt, synthetic construct
  source 1..21: mol_type = other RNA
  modified_base 1..2: mod_base = OTHER; note; note (original language) = 3'-phosphorothioate
  modified_base 19..20: mod_base = OTHER; note; note (original language) = 3'-phosphorothioate
  modified_base 1: mod_base = OTHER; note; note (original language) = 2'-methoxy
  modified_base 3..5: mod_base = OTHER; note; note (original language) = 2'-methoxy
  modified_base 7: mod_base = OTHER; note; note (original language) = 2'-methoxy
  modified_base 9..11: mod_base = OTHER; note; note (original language) = 2'-methoxy
  modified_base 13: mod_base = OTHER; note; note (original language) = 2'-methoxy
  modified_base 15: mod_base = OTHER; note; note (original language) = 2'-methoxy
  modified_base 17: mod_base = OTHER; note; note (original language) = 2'-methoxy
  modified_base 19..21: mod_base = OTHER; note; note (original language) = 2'-methoxy
  modified_base 2: mod_base = OTHER; note; note (original language) = 2'-deoxy-2'-fluoro
  modified_base 6: mod_base = OTHER; note; note (original language) = 2'-deoxy-2'-fluoro
  modified_base 8: mod_base = OTHER; note; note (original language) = 2'-deoxy-2'-fluoro
  modified_base 12: mod_base = OTHER; note; note (original language) = 2'-deoxy-2'-fluoro
  modified_base 14: mod_base = OTHER; note; note (original language) = 2'-deoxy-2'-fluoro
  modified_base 16: mod_base = OTHER; note; note (original language) = 2'-deoxy-2'-fluoro
  modified_base 19: mod_base = OTHER; note; note (original language) = 2'-deoxy-2'-fluoro
  modified_base 17: mod_base = OTHER; note; note (original language) = N=hypoxanthine
tagcgaagtgcacacgntccg

SEQ ID NO: 51 - RNA, 21 nt, synthetic construct
  source 1..21: mol_type = other RNA
  modified_base 2: mod_base = OTHER; note; note (original language) = 3'-phosphorothioate
  modified_base 19..20: mod_base = OTHER; note; note (original language) = 3'-phosphorothioate
  modified_base 2: mod_base = OTHER; note; note (original language) = 2'-deoxy-2'-fluoro
  modified_base 6: mod_base = OTHER; note; note (original language) = 2'-deoxy-2'-fluoro
  modified_base 8: mod_base = OTHER; note; note (original language) = 2'-deoxy-2'-fluoro
  modified_base 12: mod_base = OTHER; note; note (original language) = 2'-deoxy-2'-fluoro
  modified_base 14: mod_base = OTHER; note; note (original language) = 2'-deoxy-2'-fluoro
  modified_base 16: mod_base = OTHER; note; note (original language) = 2'-deoxy-2'-fluoro
  modified_base 18: mod_base = OTHER; note; note (original language) = 2'-deoxy-2'-fluoro
  modified_base 1: mod_base = OTHER; note; note (original language) = 2'-methoxy
  modified_base 3..5: mod_base = OTHER; note; note (original language) = 2'-methoxy
  modified_base 7: mod_base = OTHER; note; note (original language) = 2'-methoxy
  modified_base 9..11: mod_base = OTHER; note; note (original language) = 2'-methoxy
  modified_base 13: mod_base = OTHER; note; note (original language) = 2'-methoxy
  modified_base 15: mod_base = OTHER; note; note (original language) = 2'-methoxy
  modified_base 17: mod_base = OTHER; note; note (original language) = 2'-methoxy
  modified_base 19..21: mod_base = OTHER; note; note (original language) = 2'-methoxy
  modified_base 1: mod_base = OTHER; note; note (original language) = 5'-vinylphosphonate
  modified_base 17: mod_base = OTHER; note; note (original language) = N=hypoxanthine
tagcgaagtgcacacgntccg

SEQ ID NO: 52 - RNA, 19 nt, synthetic construct
  source 1..19: mol_type = other RNA
  modified_base 1..2: mod_base = OTHER; note; note (original language) = 3'-phosphorothioate
  modified_base 1..6: mod_base = OTHER; note; note (original language) = 2'-methoxy
  modified_base 8: mod_base = OTHER; note; note (original language) = 2'-methoxy
  modified_base 11..19: mod_base = OTHER; note; note (original language) = 2'-methoxy
  modified_base 7: mod_base = OTHER; note; note (original language) = 2'-deoxy-2'-fluoro
  modified_base 9..10: mod_base = OTHER; note; note (original language) = 2'-deoxy-2'-fluoro
gaccgtgtgcacttcgcta